European Patent Application EP 4 520 769 A1, published March 12, 2025. Title: Anti-PD-1 monoclonal antibody, derivative thereof and use thereof. Applicant: Biotheus Inc. Application EP 23778441.8 - 1111 PCT/CN2023085413, filed March 31, 2023. The sequence listing filed with the application follows.

SEQUENCE LISTING (24 sequences)

SEQ ID NO: 1 - protein, 120 aa, synthetic construct
  source 1..120: note = ADI-54872 VH
QVQLVQSGAEVKKPGASVKVSCKASGYTFTEYYIYWVRQAPGQGLEWIGGINPSNGGTNFNEKFKPRVTMTVDTSTSTAYMELSSLRSEDTAVYYCTVRDFRFDKGFKYWGQGTLVTVSS

SEQ ID NO: 2 - protein, 111 aa, synthetic construct
  source 1..111: note = ADI-54872 VL
EIVLTQSPATLSLSPGERATLSCRASKSVSTSGLNYVHWYQRKPGQAPRLLIYLGSYLDSGVPARFSGSGSGTDFTLTISSLEPEDFAVYYCQQSWELPLTFGGGTKVEIK

SEQ ID NO: 3 - protein, 120 aa, synthetic construct
  source 1..120: note = ADI-54872-1 VH
QVQLVQSGAEVKKPGASVKVSCKASGYTFTEYYIYWVRQAPGQCLEWIGGINPSNGGTNFNEKFKPRVTMTVDTSTSTAYMELSSLRSEDTAVYYCTVRDFRFDKGFKYWGQGTLVTVSS

SEQ ID NO: 4 - protein, 111 aa, synthetic construct
  source 1..111: note = ADI-54872-1 VL
EIVLTQSPATLSLSPGERATLSCRASKSVSTSGLNYVHWYQRKPGQAPRLLIYLGSYLDSGVPARFSGSGSGTDFTLTISSLEPEDFAVYYCQQSWELPLTFGCGTKVEIK

SEQ ID NO: 5 - protein, 120 aa, synthetic construct
  source 1..120: note = ADI-63628 VH
QVQLVQSGAEVKKPGASVKVSCKASGFTFTEYYIYWVRQAPGQCLEWIGGINPSNGGTNFNEKFKPRVTMTVDTSTSTAYMELSSLRSEDTAVYYCTVRDFRFDKGFKYWGQGTLVTVSS

SEQ ID NO: 6 - protein, 111 aa, synthetic construct
  source 1..111: note = ADI-63628 VL
EIVLTQSPATLSLSPGERATLSCRASKSVSTSGLNYVHWYQRKPGQAPRLLIYLGSYRDSGVPARFSGSGSGTDFTLTISSLEPEDFAVYYCQQSWELPLTFGCGTKVEIK

SEQ ID NO: 7 - protein, 9 aa, synthetic construct
  source 1..9: note = ADI-54872/ADI-54872-1 HCDR-1
YTFTEYYIY

SEQ ID NO: 8 - protein, 17 aa, synthetic construct
  source 1..17: note = ADI-54872/ADI-54872-1/ADI-63628 HCDR-2
GINPSNGGTNFNEKFKP

SEQ ID NO: 9 - protein, 13 aa, synthetic construct
  source 1..13: note = ADI-54872/ADI-54872-1/ADI-63628 HCDR-3
TVRDFRFDKGFKY

SEQ ID NO: 10 - protein, 15 aa, synthetic construct
  source 1..15: note = ADI-54872/ADI-54872-1/ADI-63628 LCDR-1
RASKSVSTSGLNYVH

SEQ ID NO: 11 - protein, 7 aa, synthetic construct
  source 1..7: note = ADI-54872/ADI-54872-1 LCDR-2
LGSYLDS

SEQ ID NO: 12 - protein, 9 aa, synthetic construct
  source 1..9: note = ADI-54872/ADI-54872-1/ADI-63628 LCDR-3
QQSWELPLT

SEQ ID NO: 13 - protein, 9 aa, synthetic construct
  source 1..9: note = ADI-63628 HCDR-1
FTFTEYYIY

SEQ ID NO: 14 - protein, 7 aa, synthetic construct
  source 1..7: note = ADI-63628 LCDR-2
LGSYRDS

SEQ ID NO: 15 - protein, 329 aa, synthetic construct
  source 1..329: note = Human IgG1 LALA heavy chain constant region
ASTKGPSVFPLAPSSKSTSGGTAALGCLVKDYFPEPVTVSWNSGALTSGVHTFPAVLQSSGLYSLSSVVTVPSSSLGTQTYICNVNHKPSNTKVDKKVEPKSCDKTHTCPPCPAPEAAGGPSVFLFPPKPKDTLMISRTPEVTCVVVDVSHEDPEVKFNWYVDGVEVHNAKTKPREEQYNSTYRVVSVLTVLHQDWLNGKEYKCKVSNKALPAPIEKTISKAKGQPREPQVYTLPPSRDELTKNQVSLTCLVKGFYPSDIAVEWESNGQPENNYKTTPPVLDSDGSFFLYSKLTVDKSRWQQGNVFSCSVMHEALHNHYTQKSLSLSPG

SEQ ID NO: 16 - protein, 107 aa, synthetic construct [sequence omitted]

SEQ ID NO: 17 - protein, 606 aa, synthetic construct
  source 1..606: note = 54872-TGF-betaRII heavy chain
QVQLVQSGAEVKKPGASVKVSCKASGYTFTEYYIYWVRQAPGQGLEWIGGINPSNGGTNFNEKFKPRVTMTVDTSTSTAYMELSSLRSEDTAVYYCTVRDFRFDKGFKYWGQGTLVTVSSASTKGPSVFPLAPSSKSTSGGTAALGCLVKDYFPEPVTVSWNSGALTSGVHTFPAVLQSSGLYSLSSVVTVPSSSLGTQTYICNVNHKPSNTKVDKKVEPKSCDKTHTCPPCPAPEAAGGPSVFLFPPKPKDTLMISRTPEVTCVVVDVSHEDPEVKFNWYVDGVEVHNAKTKPREEQYNSTYRVVSVLTVLHQDWLNGKEYKCKVSNKALPAPIEKTISKAKGQPREPQVYTLPPSRDELTKNQVSLTCLVKGFYPSDIAVEWESNGQPENNYKTTPPVLDSDGSFFLYSKLTVDKSRWQQGNVFSCSVMHEALHNHYTQKSLSLSPGGGGGAGGGGAGGGGAGGGGAGIPPHVQKSVNNDMIVTDNNGAVKFPQLCKFCDVRFSTCDNQKSCMSNCSITSICEKPQEVCVAVWRKNDENITLETVCHDPKLPYHDFILEDAASPKCIMKEKKKPGETFFMCSCSSDECNDNIIFSEEYNTSNPD

SEQ ID NO: 18 - protein, 218 aa, synthetic construct
  source 1..218: note = 54872-TGF-betaRII light chain
EIVLTQSPATLSLSPGERATLSCRASKSVSTSGLNYVHWYQRKPGQAPRLLIYLGSYLDSGVPARFSGSGSGTDFTLTISSLEPEDFAVYYCQQSWELPLTFGGGTKVEIKRTVAAPSVFIFPPSDEQLKSGTASVVCLLNNFYPREAKVQWKVDNALQSGNSQESVTEQDSKDSTYSLSSTLTLSKADYEKHKVYACEVTHQGLSSPVTKSFNRGEC

SEQ ID NO: 19 - protein, 136 aa, synthetic construct
  source 1..136: note = TGF-betaRII extracellular region
IPPHVQKSVNNDMIVTDNNGAVKFPQLCKFCDVRFSTCDNQKSCMSNCSITSICEKPQEVCVAVWRKNDENITLETVCHDPKLPYHDFILEDAASPKCIMKEKKKPGETFFMCSCSSDECNDNIIFSEEYNTSNPD

SEQ ID NO: 20 - protein, 147 aa, synthetic construct
  source 1..147: note = Human PD-1 ECD
FLDSPDRPWNPPTFSPALLVVTEGDNATFTCSFSNTSESFVLNWYRMSPSNQTDKLAAFPEDRSQPGQDCRFRVTQLPNGRDFHMSVVRARRNDSGTYLCGAISLAPKAQIKESLRAELRVTERRAEVPTAHPSPSPRPAGQFQTLV

SEQ ID NO: 21 - protein, 165 aa, synthetic construct
  source 1..165: note = Cynomolgus monkey PD-1 ECD
MQIPQAPWPVVWAVLQLGWRPGWFLESPDRPWNAPTFSPALLLVTEGDNATFTCSFSNASESFVLNWYRMSPSNQTDKLAAFPEDRSQPGQDCRFRVTRLPNGRDFHMSVVRARRNDSGTYLCGAISLAPKAQIKESLRAELRVTERRAEVPTAHPSPSPRPAGQ

SEQ ID NO: 22 - protein, 226 aa, synthetic construct
  source 1..226: note = IgG1 CH2/CH3-LALA constant region sequence (Fc)
DKTHTCPPCPAPELLGGPSVFLFPPKPKDTLMISRTPEVTCVVVDVSHEDPEVKFNWYVDGVEVHNAKTKPREEQYNSTYRVVSVLTVLHQDWLNGKEYKCKVSNKALPAPIEKTISKAKGQPREPQVYTLPPSRDELTKNQVSLTCLVKGFYPSDIAVEWESNGQPENNYKTTPPVLDSDGSFFLYSKLTVDKSRWQQGNVFSCSVMHEALHNHYTQKSLSLSPG

SEQ ID NO: 23 - protein, 487 aa, synthetic construct
  source 1..487: note = ADI-54872-1 full-length sequence
DKTHTCPPCPAPELLGGPSVFLFPPKPKDTLMISRTPEVTCVVVDVSHEDPEVKFNWYVDGVEVHNAKTKPREEQYNSTYRVVSVLTVLHQDWLNGKEYKCKVSNKALPAPIEKTISKAKGQPREPQVYTLPPSRDELTKNQVSLTCLVKGFYPSDIAVEWESNGQPENNYKTTPPVLDSDGSFFLYSKLTVDKSRWQQGNVFSCSVMHEALHNHYTQKSLSLSPGGGGGSGGGGSQVQLVQSGAEVKKPGASVKVSCKASGYTFTEYYIYWVRQAPGQCLEWIGGINPSNGGTNFNEKFKPRVTMTVDTSTSTAYMELSSLRSEDTAVYYCTVRDFRFDKGFKYWGQGTLVTVSSGGGGSGGGGSGGGGSGGGGSEIVLTQSPATLSLSPGERATLSCRASKSVSTSGLNYVHWYQRKPGQAPRLLIYLGSYLDSGVPARFSGSGSGTDFTLTISSLEPEDFAVYYCQQSWELPLTFGCGTKVEIK

SEQ ID NO: 24 - protein, 487 aa, synthetic construct
  source 1..487: note = ADI-63628 full-length sequence
DKTHTCPPCPAPELLGGPSVFLFPPKPKDTLMISRTPEVTCVVVDVSHEDPEVKFNWYVDGVEVHNAKTKPREEQYNSTYRVVSVLTVLHQDWLNGKEYKCKVSNKALPAPIEKTISKAKGQPREPQVYTLPPSRDELTKNQVSLTCLVKGFYPSDIAVEWESNGQPENNYKTTPPVLDSDGSFFLYSKLTVDKSRWQQGNVFSCSVMHEALHNHYTQKSLSLSPGGGGGAGGGGAQVQLVQSGAEVKKPGASVKVSCKASGFTFTEYYIYWVRQAPGQCLEWIGGINPSNGGTNFNEKFKPRVTMTVDTSTSTAYMELSSLRSEDTAVYYCTVRDFRFDKGFKYWGQGTLVTVSSGGGGSGGGGSGGGGSGGGGSEIVLTQSPATLSLSPGERATLSCRASKSVSTSGLNYVHWYQRKPGQAPRLLIYLGSYRDSGVPARFSGSGSGTDFTLTISSLEPEDFAVYYCQQSWELPLTFGCGTKVEIK